European Patent Specification EP 3 512 877 B1, published March 26, 2025. Title: Nidogen-1 Assay. Applicant: Nordic Bioscience A/S. The sequence listing filed with the application follows.

SEQUENCE LISTING (16 sequences)

SEQ ID NO: 1 - protein, 6 aa, Artificial Sequence
  C-terminal neo-epitope
CQHERE

SEQ ID NO: 2 - protein, 6 aa, Artificial Sequence
  C-terminal neo-epitope
YSLLPL

SEQ ID NO: 3 - protein, 6 aa, Artificial Sequence
  C-terminal neo-epitope
IIRQDL

SEQ ID NO: 4 - protein, 6 aa, Artificial Sequence
  N-terminal neo-epitope
APVGGI

SEQ ID NO: 5 - protein, 6 aa, Artificial Sequence
  N-terminal neo-epitope
HILGAA

SEQ ID NO: 6 - protein, 6 aa, Artificial Sequence
  N-terminal neo-epitope
GSPEGI

SEQ ID NO: 7 - protein, 11 aa, Artificial Sequence
  C-terminal neo-epitope
VEKTRCQHERE

SEQ ID NO: 8 - protein, 10 aa, Artificial Sequence
  Truncated C-terminal neo-epitope sequence
VEKTRCQHER

SEQ ID NO: 9 - protein, 12 aa, Artificial Sequence
  elongated C-terminal neo-epitope sequence
VEKTRCQHEREH

SEQ ID NO: 10 - protein, 11 aa, Artificial Sequence
  SITE 1: N-terminal biotinylated with optional linker between N-terminus and biotin residue
  Screening peptide
VEKTRCQHERE

SEQ ID NO: 11 - protein, 11 aa, Artificial Sequence
  Selection peptide
VEKTRCQHERE

SEQ ID NO: 12 - protein, 10 aa, Artificial Sequence
  nonsense peptide
APVGGIIGWM

SEQ ID NO: 13 - protein, 10 aa, Artificial Sequence
  SITE 1: N-terminal biotinylated with optional linker between N-terminus and biotin residue
  nonsense screening peptide
APVGGIIGWM

SEQ ID NO: 14 - protein, 11 aa, Artificial Sequence
  SITE 1: Keyhole Limpet Hemocyanin attached to N-terminus
  immunogenic peptide
VEKTRCQHERE

SEQ ID NO: 15 - protein, 11 aa, Artificial Sequence
  truncated selection peptide
EVEKTRCQHER

SEQ ID NO: 16 - protein, 12 aa, Artificial Sequence
  elongated selection peptide
VEKTRCQHEREH